European Patent Specification EP 2 831 279 B1, published May 3, 2023. Title: RAPID ANEUPLOIDY DETECTION. Applicant: VOGELSTEIN, Bert KINZLER,  Kenneth W. PAPADOPOULOS, Nickolas KINDE, Isaac. The sequence listing filed with the application follows.

SEQUENCE LISTING (14 sequences)

SEQ ID NO: 1 - DNA, 18 bp, Artificial Sequence
  oligonucleotide primers
acacagggaggggaacat

SEQ ID NO: 2 - DNA, 17 bp, Artificial Sequence
  oligonucleotide primers
tgccatggtggtttgct

SEQ ID NO: 3 - DNA, 18 bp, Artificial Sequence
  oligonucleotide primers
acacagggaggggaacat

SEQ ID NO: 4 - DNA, 55 bp, Artificial Sequence
  oligonucleotide primers
  misc_feature (1)...(55): n = A,T,C or G
cgacgtaaaacgacggccagtnnnnnnnnnnnnnnnnacacagggaggggaacat

SEQ ID NO: 5 - DNA, 59 bp, Artificial Sequence
  oligonucleotide primers
cgacgtaaaacgacggccagthbvdhbvdhbvdhbvdhbvdacacagggaggggaacat

SEQ ID NO: 6 - DNA, 42 bp, Artificial Sequence
  oligonucleotide primers
cacacaggaaacagctatgaccatgtgccatggtggtttgct

SEQ ID NO: 7 - DNA, 50 bp, Artificial Sequence
  oligonucleotide primers
aatgatacggcgaccaccgagatctacaccgacgtaaaacgacggccagt

SEQ ID NO: 8 - DNA, 55 bp, Artificial Sequence
  oligonucleotide primers
caagcagaagacggcatacgagatgatcagcacacaggaaacagctatgaccatg

SEQ ID NO: 9 - DNA, 55 bp, Artificial Sequence
  oligonucleotide primers
caagcagaagacggcatacgagatgccaatcacacaggaaacagctatgaccatg

SEQ ID NO: 10 - DNA, 55 bp, Artificial Sequence
  oligonucleotide primers
caagcagaagacggcatacgagattgaccacacacaggaaacagctatgaccatg

SEQ ID NO: 11 - DNA, 55 bp, Artificial Sequence
  oligonucleotide primers
caagcagaagacggcatacgagatttaggccacacaggaaacagctatgaccatg

SEQ ID NO: 12 - DNA, 55 bp, Artificial Sequence
  oligonucleotide primers
caagcagaagacggcatacgagatcttgtacacacaggaaacagctatgaccatg

SEQ ID NO: 13 - DNA, 32 bp, Artificial Sequence
  oligonucleotide primers
gagatctacaccgacgtaaaacgacggccagt

SEQ ID NO: 14 - DNA, 25 bp, Artificial Sequence
  oligonucleotide primers
catggtcatagctgtttcctgtgtg